European Patent Application EP 4 684 797 A2, published January 28, 2026. Title: STABLE PROTEIN SOLUTION FORMULATION CONTAINING HIGH CONCENTRATION OF AN ANTI-VEGF ANTIBODY. Applicant: Novartis AG. Application WO PCT/US2015/059571, filed November 6, 2015. The sequence listing filed with the application follows.

SEQUENCE LISTING (10 sequences)

SEQ ID NO: 1 - protein, 120 aa, synthetic construct
  REGION 1..120: note = Synthetic heavy chain
EVQLVESGGGLVQPGGSLRLSCTASGFSLTDYYYMTWVRQAPGKGLEWVGFIDPDDDPYYATWAKGRFTISRDNSKNTLYLQMNSLRAEDTAVYYCAGGDHNSGWGLDIWGQGTLVTVSS

SEQ ID NO: 2 - protein, 111 aa, synthetic construct
  REGION 1..111: note = Synthetic light chain
EIVMTQSPSTLSASVGDRVIITCQASEIIHSWLAWYQQKPGKAPKLLIYLASTLASGVPSRFSGSGSGAEFTLTISSLQPDDFATYYCQNVYLASTNGANFGQGTKLTVLG

SEQ ID NO: 3 - protein, 251 aa, synthetic construct
  REGION 1..251: note = Synthetic antibody construct
EIVMTQSPSTLSASVGDRVIITCQASEIIHSWLAWYQQKPGKAPKLLIYLASTLASGVPSRFSGSGSGAEFTLTISSLQPDDFATYYCQNVYLASTNGANFGQGTKLTVLGGGGGSGGGGSGGGGSGGGGSEVQLVESGGGLVQPGGSLRLSCTASGFSLTDYYYMTWVRQAPGKGLEWVGFIDPDDDPYYATWAKGRFTISRDNSKNTLYLQMNSLRAEDTAVYYCAGGDHNSGWGLDIWGQGTLVTVSS

SEQ ID NO: 4 - protein, 252 aa, synthetic construct
  REGION 1..252: note = Synthetic antibody construct
MEIVMTQSPSTLSASVGDRVIITCQASEIIHSWLAWYQQKPGKAPKLLIYLASTLASGVPSRFSGSGSGAEFTLTISSLQPDDFATYYCQNVYLASTNGANFGQGTKLTVLGGGGGSGGGGSGGGGSGGGGSEVQLVESGGGLVQPGGSLRLSCTASGFSLTDYYYMTWVRQAPGKGLEWVGFIDPDDDPYYATWAKGRFTISRDNSKNTLYLQMNSLRAEDTAVYYCAGGDHNSGWGLDIWGQGTLVTVSS

SEQ ID NO: 5 - protein, 11 aa, synthetic construct
  REGION 1..11: note = CDR H1
GFSLTDYYYMT

SEQ ID NO: 6 - protein, 16 aa, synthetic construct
  REGION 1..16: note = CDR H2
FIDPDDDPYYATWAKG

SEQ ID NO: 7 - protein, 11 aa, synthetic construct
  REGION 1..11: note = CDR H3
GDHNSGWGLDI

SEQ ID NO: 8 - protein, 11 aa, synthetic construct
  REGION 1..11: note = CDR L1
QASEIIHSWLA

SEQ ID NO: 9 - protein, 7 aa, synthetic construct
  REGION 1..7: note = CDR L2
LASTLAS

SEQ ID NO: 10 - protein, 12 aa, synthetic construct
  REGION 1..12: note = CDR L3
QNVYLASTNGAN